European Patent Specification EP 3 401 334 B1, published February 15, 2023. Title: MONOCLONAL ANTIBODIES AGAINST CLAUDIN-18 FOR TREATMENT OF CANCER. Applicant: Ganymed Pharmaceuticals GmbH et al. The sequence listing filed with the application follows.

SEQUENCE LISTING (157 sequences)

SEQ ID NO: 1 - DNA, 786 bp, Homo sapiens
atggccgtgactgcctgtcagggcttggggttcgtggtttcactgattgggattgcgggcatcattgctgccacctgcatggaccagtggagcacccaagacttgtacaacaaccccgtaacagctgttttcaactaccaggggctgtggcgctcctgtgtccgagagagctctggcttcaccgagtgccggggctacttcaccctgctggggctgccagccatgctgcaggcagtgcgagccctgatgatcgtaggcatcgtcctgggtgccattggcctcctggtatccatctttgccctgaaatgcatccgcattggcagcatggaggactctgccaaagccaacatgacactgacctccgggatcatgttcattgtctcaggtctttgtgcaattgctggagtgtctgtgtttgccaacatgctggtgactaacttctggatgtccacagctaacatgtacaccggcatgggtgggatggtgcagactgttcagaccaggtacacatttggtgcggctctgttcgtgggctgggtcgctggaggcctcacactaattgggggtgtgatgatgtgcatcgcctgccggggcctggcaccagaagaaaccaactacaaagccgtttcttatcatgcctcgggccacagtgttgcctacaagcctggaggcttcaaggccagcactggctttgggtccaacaccaaaaacaagaagatatacgatggaggtgcccgcacagaggacgaggtacaatcttatccttccaagcacgactatgtgtaa

SEQ ID NO: 2 - protein, 261 aa, Homo sapiens
MAVTACQGLGFVVSLIGIAGIIAATCMDQWSTQDLYNNPVTAVFNYQGLWRSCVRESSGFTECRGYFTLLGLPAMLQAVRALMIVGIVLGAIGLLVSIFALKCIRIGSMEDSAKANMTLTSGIMFIVSGLCAIAGVSVFANMLVTNFWMSTANMYTGMGGMVQTVQTRYTFGAALFVGWVAGGLTLIGGVMMCIACRGLAPEETNYKAVSYHASGHSVAYKPGGFKASTGFGSNTKNKKIYDGGARTEDEVQSYPSKHDYV

SEQ ID NO: 3 - DNA, 816 bp, Homo sapiens
atggccgtgactgcctgtcagggcttggggttcgtggtttcactgattgggattgcgggcatcattgctgccacctgcatggaccagtggagcacccaagacttgtacaacaaccccgtaacagctgttttcaactaccaggggctgtggcgctcctgtgtccgagagagctctggcttcaccgagtgccggggctacttcaccctgctggggctgccagccatgctgcaggcagtgcgagccctgatgatcgtaggcatcgtcctgggtgccattggcctcctggtatccatctttgccctgaaatgcatccgcattggcagcatggaggactctgccaaagccaacatgacactgacctccgggatcatgttcattgtctcaggtctttgtgcaattgctggagtgtctgtgtttgccaacatgctggtgactaacttctggatgtccacagctaacatgtacaccggcatgggtgaacaaaaactcatctcagaagaggatctggggatggtgcagactgttcagaccaggtacacatttggtgcggctctgttcgtgggctgggtcgctggaggcctcacactaattgggggtgtgatgatgtgcatcgcctgccggggcctggcaccagaagaaaccaactacaaagccgtttcttatcatgcctcgggccacagtgttgcctacaagcctggaggcttcaaggccagcactggctttgggtccaacaccaaaaacaagaagatatacgatggaggtgcccgcacagaggacgaggtacaatcttatccttccaagcacgactatgtgtaa

SEQ ID NO: 4 - protein, 271 aa, Homo sapiens
MAVTACQGLGFVVSLIGIAGIIAATCMDQWSTQDLYNNPVTAVFNYQGLWRSCVRESSGFTECRGYFTLLGLPAMLQAVRALMIVGIVLGAIGLLVSIFALKCIRIGSMEDSAKANMTLTSGIMFIVSGLCAIAGVSVFANMLVTNFWMSTANMYTGMGEQKLISEEDLGMVQTVQTRYTFGAALFVGWVAGGLTLIGGVMMCIACRGLAPEETNYKAVSYHASGHSVAYKPGGFKASTGFGSNTKNKKIYDGGARTEDEVQSYPSKHDYV

SEQ ID NO: 5 - DNA, 813 bp, Homo sapiens
atggccgtgactgcctgtcagggcttggggttcgtggtttcactgattgggattgcgggcatcattgctgccacctgcatggaccagtggagcacccaagacttgtacaacaaccccgtaacagctgttttcaactaccaggggctgtggcgctcctgtgtccgagagagctctggcttcaccgagtgccggggctacttcaccctgtacccatacgacgtgccagactacgcactggggctgccagccatgctgcaggcagtgcgagccctgatgatcgtaggcatcgtcctgggtgccattggcctcctggtatccatctttgccctgaaatgcatccgcattggcagcatggaggactctgccaaagccaacatgacactgacctccgggatcatgttcattgtctcaggtctttgtgcaattgctggagtgtctgtgtttgccaacatgctggtgactaacttctggatgtccacagctaacatgtacaccggcatgggtgggatggtgcagactgttcagaccaggtacacatttggtgcggctctgttcgtgggctgggtcgctggaggcctcacactaattgggggtgtgatgatgtgcatcgcctgccggggcctggcaccagaagaaaccaactacaaagccgtttcttatcatgcctcgggccacagtgttgcctacaagcctggaggcttcaaggccagcactggctttgggtccaacaccaaaaacaagaagatatacgatggaggtgcccgcacagaggacgaggtacaatcttatccttccaagcacgactatgtgtaa

SEQ ID NO: 6 - protein, 270 aa, Homo sapiens
MAVTACQGLGFVVSLIGIAGIIAATCMDQWSTQDLYNNPVTAVFNYQGLWRSCVRESSGFTECRGYFTLYPYDVPDYALGLPAMLQAVRALMIVGIVLGAIGLLVSIFALKCIRIGSMEDSAKANMTLTSGIMFIVSGLCAIAGVSVFANMLVTNFWMSTANMYTGMGGMVQTVQTRYTFGAALFVGWVAGGLTLIGGVMMCIACRGLAPEETNYKAVSYHASGHSVAYKPGGFKASTGFGSNTKNKKIYDGGARTEDEVQSYPSKHDYV

SEQ ID NO: 7 - DNA, 786 bp, Homo sapiens
atgtccaccaccacatgccaagtggtggcgttcctcctgtccatcctggggctggccggctgcatcgcggccaccgggatggacatgtggagcacccaggacctgtacgacaaccccgtcacctccgtgttccagtacgaagggctctggaggagctgcgtgaggcagagttcaggcttcaccgaatgcaggccctatttcaccatcctgggacttccagccatgctgcaggcagtgcgagccctgatgatcgtaggcatcgtcctgggtgccattggcctcctggtatccatctttgccctgaaatgcatccgcattggcagcatggaggactctgccaaagccaacatgacactgacctccgggatcatgttcattgtctcaggtctttgtgcaattgctggagtgtctgtgtttgccaacatgctggtgactaacttctggatgtccacagctaacatgtacaccggcatgggtgggatggtgcagactgttcagaccaggtacacatttggtgcggctctgttcgtgggctgggtcgctggaggcctcacactaattgggggtgtgatgatgtgcatcgcctgccggggcctggcaccagaagaaaccaactacaaagccgtttcttatcatgcctcaggccacagtgttgcctacaagcctggaggcttcaaggccagcactggctttgggtccaacaccaaaaacaagaagatatacgatggaggtgcccgcacagaggacgaggtacaatcttatccttccaagcacgactatgtgtaa

SEQ ID NO: 8 - protein, 261 aa, Homo sapiens
MSTTTCQVVAFLLSILGLAGCIAATGMDMWSTQDLYDNPVTSVFQYEGLWRSCVRQSSGFTECRPYFTILGLPAMLQAVRALMIVGIVLGAIGLLVSIFALKCIRIGSMEDSAKANMTLTSGIMFIVSGLCAIAGVSVFANMLVTNFWMSTANMYTGMGGMVQTVQTRYTFGAALFVGWVAGGLTLIGGVMMCIACRGLAPEETNYKAVSYHASGHSVAYKPGGFKASTGFGSNTKNKKIYDGGARTEDEVQSYPSKHDYV

SEQ ID NO: 9 - DNA, 795 bp, Mus musculus
atggccaccaccacgtgccaggtggtagggcttctcctgtccctcctgggtctggccggctgcatagccgccactgggatggacatgtggagcactcaagacctgtatgacaacccagtcaccgccgtgttccagtatgaagggctctggaggagttgcgtgcaacagagctcggggttcaccgagtgccggccatacttcaccatcctgggccttccagccatgctgcaagctgtacgagccctgatgatcgtgggcattgttctgggggtcatcggtatcctcgtgtccatcttcgccctgaagtgcattcgcattggtagcatggatgactctgccaaggccaagatgactctgacttctgggatcttgttcatcatctccggcatctgtgcaatcattggtgtgtctgtgtttgccaacatgctggtgaccaacttctggatgtccacagctaacatgtacagcggcatgggcggcatgggtggcatggtgcagaccgttcagaccaggtacacctttggtgcagctctgttcgtgggctgggttgctggaggcctcaccctgattgggggagtgatgatgtgcatcgcctgccgtggcctgacaccagatgacagcaacttcaaagctgtgtcttaccatgcctctggccaaaatgttgcctacaggcctggaggctttaaggccagcactggctttgggtccaacaccagaaacaagaagatctacgatgggggtgcccgcacagaagacgatgaacagtctcatcctaccaagtatgactatgtgtag

SEQ ID NO: 10 - DNA, 795 bp, Mus musculus
atgtcggtgaccgcctgccagggcttggggtttgtggtgtcactgatcgggtttgcgggcatcattgcagccacttgtatggaccagtggagcacccaggatttatacaacaacccggtgaccgctgtattcaactaccaagggctatggcgttcatgcgtccgagagagctctggcttcaccgagtgccgaggctacttcaccctgttggggttgccagccatgctgcaagctgtacgagccctgatgatcgtgggcattgttctgggggtcatcggtatcctcgtgtccatcttcgccctgaagtgcattcgcattggtagcatggatgactctgccaaggccaagatgactctgacttctgggatcttgttcatcatctccggcatctgtgcaatcattggtgtgtctgtgtttgccaacatgctggtgaccaacttctggatgtccacagctaacatgtacagcggcatgggcggcatgggtggcatggtgcagaccgttcagaccaggtacacctttggtgcagctctgttcgtgggctgggttgctggaggcctcaccctgattgggggagtgatgatgtgcatcgcctgccgtggcctgacaccagatgacagcaacttcaaagctgtgtcttaccatgcctctggccaaaatgttgcctacaggcctggaggctttaaggccagcactggctttgggtccaacaccagaaacaagaagatctacgatgggggtgcccgcacagaagacgatgaacagtctcatcctaccaagtatgactatgtgtag

SEQ ID NO: 11 - DNA, 21 bp, Artificial
  Description of artificial sequence: Oligonucleotide
tggctctgtgtcgacactgtg

SEQ ID NO: 12 - DNA, 21 bp, Artificial
  Description of artificial sequence: Oligonucleotide
gtgtacatgttagctgtggac

SEQ ID NO: 13 - protein, 55 aa, Homo sapiens
MDMWSTQDLYDNPVTSVFQYEGLWRSCVRQSSGFTECRPYFTILGLPAMLQAVRA

SEQ ID NO: 14 - protein, 153 aa, Homo sapiens
MDMWSTQDLYDNPVTSVFQYEGLWRSCVRQSSGFTECRPYFTILGLPAMLQAVRALMIVGIVLGAIGLLVSIFALKCIRIGSMEDSAKANMTLTSGIMFIVSGLCAIAGVSVFANMLVTNFWMSTANMYTGMGGMVQTVQTRYTFGAALFVGW

SEQ ID NO: 15 - DNA, 390 bp, Homo sapiens
atggagacagacacactcctgctatgggtactgctgctctgggttccaggttccactggtgacgcggcccagccggccaggcgcgcgcgccgtacgaagcttggtaccgagctcggatccactccagtgtggtggaattctgcagatggccgcatggaccagtggagcacccaagacttgtacaacaaccccgtaacagctgttttcaactaccaggggctgtggcgctcctgtgtccgagagagctctggcttcaccgagtgccggggctacttcaccctgctggggctgccagccatgctgcaggcagtgcgagcggccatccagcacagtggcggccgctcgaggagggcccgaacaaaaactcatctcagaagaggatctgaatag

SEQ ID NO: 16 - protein, 129 aa, Homo sapiens
METDTLLLWVLLLWVPGSTGDAAQPARRARRTKLGTELGSTPVWWNSADGRMDQWSTQDLYNNPVTAVFNYQGLWRSCVRESSGFTECRGYFTLLGLPAMLQAVRAAIQHSGGRSRRARTKTHLRRGSE

SEQ ID NO: 17 - DNA, 411 bp, Homo sapiens
atggagacagacacactcctgctatgggtactgctgctctgggttccaggttccactggtgacgcggcccagccggccaggcgcgcgcgccgtacgaagcttggtaccgagctcggatccactccagtgtggtggaattctgcagatggccgcgccctgatgatcgtaggcatcgtcctgggtgccattggcctcctggtatccatctttgccctgaaatgcatccgcattggcagcatggaggactctgccaaagccaacatgacactgacatccgggatcatgttcattgtctcaggtctttgtgcaattgctggagtgtctgtgtttgccaacgcggccatccagcacagtggcggccgctcgaggagggcccgaacaaaaactcatctcagaagaggatctgaatag

SEQ ID NO: 18 - protein, 136 aa, Homo sapiens
METDTLLLWVLLLWVPGSTGDAAQPARRARRTKLGTELGSTPVWWNSADGRALMIVGIVLGAIGLLVSIFALKCIRIGSMEDSAKANMTLTSGIMFIVSGLCAIAGVSVFANAAIQHSGGRSRRARTKTHLRRGSE

SEQ ID NO: 19 - DNA, 531 bp, Homo sapiens
atggagacagacacactcctgctatgggtactgctgctctgggttccaggttccactggtgacgcggcccagccggccaggcgcgccatggaccagtggagcacccaagacttgtacaacaaccccgtaacagctgttttcaactaccaggggctgtggcgctcctgtgtccgagagagctctggcttcaccgagtgccggggctacttcaccctgctggggctgccagccatgctgcaggcagtgcgagccctgatgatcgtaggcatcgtcctgggtgccattggcctcctggtatccatctttgccctgaaatgcatccgcattggcagcatggaggactctgccaaagccaacatgacactgacctccgggatcatgttcattgtctcaggtctttgtgcaattgctggagtgtctgtgtttgccaacatgctggtgactaacttctggatgtccacagctaacatgtacaccggcatgggtgggatggtgcagactgttcagaccaggtacacatttggtgcgtag

SEQ ID NO: 20 - protein, 176 aa, Homo sapiens
METDTLLLWVLLLWVPGSTGDAAQPARRAMDQWSTQDLYNNPVTAVFNYQGLWRSCVRESSGFTECRGYFTLLGLPAMLQAVRALMIVGIVLGAIGLLVSIFALKCIRIGSMEDSAKANMTLTSGIMFIVSGLCAIAGVSVFANMLVTNFWMSTANMYTGMGGMVQTVQTRYTFGA

SEQ ID NO: 21 - protein, 10 aa, Homo sapiens
DQWSTQDLYN

SEQ ID NO: 22 - protein, 11 aa, Homo sapiens
NNPVTAVFNYQ

SEQ ID NO: 23 - protein, 14 aa, Homo sapiens
STQDLYNNPVTAVF

SEQ ID NO: 24 - protein, 12 aa, Homo sapiens
DMWSTQDLYDNP

SEQ ID NO: 25 - protein, 12 aa, Homo sapiens
CRPYFTILGLPA

SEQ ID NO: 26 - protein, 13 aa, Homo sapiens
TNFWMSTANMYTG

SEQ ID NO: 27 - protein, 13 aa, Homo sapiens
DSAKANMTLTSGI

SEQ ID NO: 28 - protein, 55 aa, Homo sapiens
MDQWSTQDLYNNPVTAVFNYQGLWRSCVRESSGFTECRGYFTLLGLPAMLQAVRA

SEQ ID NO: 29 - protein, 24 aa, Homo sapiens
FALKCIRIGSMEDSAKANMTLTSG

SEQ ID NO: 30 - protein, 40 aa, Homo sapiens
ANMLVTNFWMSTANMYTGMGGMVQTVQTRYTFGAALFVGW

SEQ ID NO: 31 - protein, 153 aa, Homo sapiens
MDQWSTQDLYNNPVTAVFNYQGLWRSCVRESSGFTECRGYFTLLGLPAMLQAVRALMIVGIVLGAIGLLVSIFALKCIRIGSMEDSAKANMTLTSGIMFIVSGLCAIAGVSVFANMLVTNFWMSTANMYTGMGGMVQTVQTRYTFGAALFVGW

SEQ ID NO: 32 - DNA, 3359 bp, Homo sapiens
cacaccttcggcagcaggagggcggcagcttctcgcaggcggcagggcgggcggccaggatcatgtccaccaccacatgccaagtggtggcgttcctcctgtccatcctggggctggccggctgcatcgcggccaccgggatggacatgtggagcacccaggacctgtacgacaaccccgtcacctccgtgttccagtacgaagggctctggaggagctgcgtgaggcagagttcaggcttcaccgaatgcaggccctatttcaccatcctgggacttccagccatgctgcaggcagtgcgagccctgatgatcgtaggcatcgtcctgggtgccattggcctcctggtatccatctttgccctgaaatgcatccgcattggcagcatggaggactctgccaaagccaacatgacactgacctccgggatcatgttcattgtctcaggtctttgtgcaattgctggagtgtctgtgtttgccaacatgctggtgactaacttctggatgtccacagctaacatgtacaccggcatgggtgggatggtgcagactgttcagaccaggtacacatttggtgcggctctgttcgtgggctgggtcgctggaggcctcacactaattgggggtgtgatgatgtgcatcgcctgccggggcctggcaccagaagaaaccaactacaaagccgtttcttatcatgcctcaggccacagtgttgcctacaagcctggaggcttcaaggccagcactggctttgggtccaacaccaaaaacaagaagatatacgatggaggtgcccgcacagaggacgaggtacaatcttatccttccaagcacgactatgtgtaatgctctaagacctctcagcacgggcggaagaaactcccggagagctcacccaaaaaacaaggagatcccatctagatttcttcttgcttttgactcacagctggaagttagaaaagcctcgatttcatctttggagaggccaaatggtcttagcctcagtctctgtctctaaatattccaccataaaacagctgagttatttatgaattagaggctatagctcacattttcaatcctctatttctttttttaaatataactttctactctgatgagagaatgtggttttaatctctctctcacattttgatgatttagacagactccccctcttcctcctagtcaataaacccattgatgatctatttcccagcttatccccaagaaaacttttgaaaggaaagagtagacccaaagatgttattttctgctgtttgaattttgtctccccacccccaacttggctagtaataaacacttactgaagaagaagcaataagagaaagatatttgtaatctctccagcccatgatctcggttttcttacactgtgatcttaaaagttaccaaaccaaagtcattttcagtttgaggcaaccaaacctttctactgctgttgacatcttcttattacagcaacaccattctaggagtttcctgagctctccactggagtcctctttctgtcgcgggtcagaaattgtccctagatgaatgagaaaattattttttttaatttaagtcctaaatatagttaaaataaataatgttttagtaaaatgatacactatctctgtgaaatagcctcacccctacatgtggatagaaggaaatgaaaaaataattgctttgacattgtctatatggtactttgtaaagtcatgcttaagtacaaattccatgaaaagctcactgatcctaattctttccctttgaggtctctatggctctgattgtacatgatagtaagtgtaagccatgtaaaaagtaaataatgtctgggcacagtggctcacgcctgtaatcctagcactttgggaggctgaggaggaaggatcacttgagcccagaagttcgagactagcctgggcaacatggagaagccctgtctctacaaaatacagagagaaaaaatcagccagtcatggtggcctacacctgtagtcccagcattccgggaggctgaggtgggaggatcacttgagcccagggaggttggggctgcagtgagccatgatcacaccactgcactccagccaggtgacatagcgagatcctgtctaaaaaaataaaaaataaataatggaacacagcaagtcctaggaagtaggttaaaactaattctttaaaaaaaaaaaaaagttgagcctgaattaaatgtaatgtttccaagtgacaggtatccacatttgcatggttacaagccactgccagttagcagtagcactttcctggcactgtggtcggttttgttttgttttgctttgtttagagacggggtctcactttccaggctggcctcaaactcctgcactcaagcaattcttctaccctggcctcccaagtagctggaattacaggtgtgcgccatcacaactagctggtggtcagttttgttactctgagagctgttcacttctctgaattcacctagagtggttggaccatcagatgtttgggcaaaactgaaagctctttgcaaccacacaccttccctgagcttacatcactgcccttttgagcagaaagtctaaattccttccaagacagtagaattccatcccagtaccaaagccagataggccccctaggaaactgaggtaagagcagtctctaaaaactacccacagcagcattggtgcaggggaacttggccattaggttattatttgagaggaaagtcctcacatcaatagtacatatgaaagtgacctccaaggggattggtgaatactcataaggatcttcaggctgaacagactatgtctggggaaagaacggattatgccccattaaataacaagttgtgttcaagagtcagagcagtgagctcagaggcccttctcactgagacagcaacatttaaaccaaaccagaggaagtatttgtggaactcactgcctcagtttgggtaaaggatgagcagacaagtcaactaaagaaaaaagaaaagcaaggaggagggttgagcaatctagagcatggagtttgttaagtgctctctggatttgagttgaagagcatccatttgagttgaaggccacagggcacaatgagctctcccttctaccaccagaaagtccctggtcaggtctcaggtagtgcggtgtggctcagctgggtttttaattagcgcattctctatccaacatttaattgtttgaaagcctccatatagttagattgtgctttgtaattttgttgttgttgctctatcttattgtatatgcattgagtattaacctgaatgttttgttacttaaatattaaaaacactgttatcctacagtt

SEQ ID NO: 33 - DNA, 849 bp, Mus musculus
gagaacctgcctgtctcttgtcctctccatttgtgtggactctgtgctccatcatgtcggtgaccgcctgccagggcttggggtttgtggtgtcactgatcgggtttgcgggcatcattgcagccacttgtatggaccagtggagcacccaggatttatacaacaacccggtgaccgctgtattcaactaccaagggctatggcgttcatgcgtccgagagagctctggcttcaccgagtgccgaggctacttcaccctgttggggttgccagccatgctgcaagctgtacgagccctgatgatcgtgggcattgttctgggggtcatcggtatcctcgtgtccatcttcgccctgaagtgcattcgcattggtagcatggatgactctgccaaggccaagatgactctgacttctgggatcttgttcatcatctccggcatctgtgcaatcattggtgtgtctgtgtttgccaacatgctggtgaccaacttctggatgtccacagctaacatgtacagcggcatgggcggcatgggtggcatggtgcagaccgttcagaccaggtacaccttcggtgcagctctgttcgtgggctgggttgctggaggcctcaccctgattgggggagtgatgatgtgcatcgcctgccgtggcctgacaccagatgacagcaacttcaaagctgtgtcttaccatgcctctggccaaaatgttgcctacaggcctggaggctttaaggccagcactggctttgggtccaacaccagaaacaagaagatctacgatgggggtgcccgcacagaagacgatgaacagtctcatcctaccaagtatgactatgtgtagt

SEQ ID NO: 34 - DNA, 3350 bp, Homo sapiens
agaattgcgctgtccacttgtcgtgtggctctgtgtcgacactgtgcgccaccatggccgtgactgcctgtcagggcttggggttcgtggtttcactgattgggattgcgggcatcattgctgccacctgcatggaccagtggagcacccaagacttgtacaacaaccccgtaacagctgttttcaactaccaggggctgtggcgctcctgtgtccgagagagctctggcttcaccgagtgccggggctacttcaccctgctggggctgccagccatgctgcaggcagtgcgagccctgatgatcgtaggcatcgtcctgggtgccattggcctcctggtatccatctttgccctgaaatgcatccgcattggcagcatggaggactctgccaaagccaacatgacactgacctccgggatcatgttcattgtctcaggtctttgtgcaattgctggagtgtctgtgtttgccaacatgctggtgactaacttctggatgtccacagctaacatgtacaccggcatgggtgggatggtgcagactgttcagaccaggtacacatttggtgcggctctgttcgtgggctgggtcgctggaggcctcacactaattgggggtgtgatgatgtgcatcgcctgccggggcctggcaccagaagaaaccaactacaaagccgtttcttatcatgcctcaggccacagtgttgcctacaagcctggaggcttcaaggccagcactggctttgggtccaacaccaaaaacaagaagatatacgatggaggtgcccgcacagaggacgaggtacaatcttatccttccaagcacgactatgtgtaatgctctaagacctctcagcacgggcggaagaaactcccggagagctcacccaaaaaacaaggagatcccatctagatttcttcttgcttttgactcacagctggaagttagaaaagcctcgatttcatctttggagaggccaaatggtcttagcctcagtctctgtctctaaatattccaccataaaacagctgagttatttatgaattagaggctatagctcacattttcaatcctctatttctttttttaaatataactttctactctgatgagagaatgtggttttaatctctctctcacattttgatgatttagacagactccccctcttcctcctagtcaataaacccattgatgatctatttcccagcttatccccaagaaaacttttgaaaggaaagagtagacccaaagatgttattttctgctgtttgaattttgtctccccacccccaacttggctagtaataaacacttactgaagaagaagcaataagagaaagatatttgtaatctctccagcccatgatctcggttttcttacactgtgatcttaaaagttaccaaaccaaagtcattttcagtttgaggcaaccaaacctttctactgctgttgacatcttcttattacagcaacaccattctaggagtttcctgagctctccactggagtcctctttctgtcgcgggtcagaaattgtccctagatgaatgagaaaattattttttttaatttaagtcctaaatatagttaaaataaataatgttttagtaaaatgatacactatctctgtgaaatagcctcacccctacatgtggatagaaggaaatgaaaaaataattgctttgacattgtctatatggtactttgtaaagtcatgcttaagtacaaattccatgaaaagctcactgatcctaattctttccctttgaggtctctatggctctgattgtacatgatagtaagtgtaagccatgtaaaaagtaaataatgtctgggcacagtggctcacgcctgtaatcctagcactttgggaggctgaggaggaaggatcacttgagcccagaagttcgagactagcctgggcaacatggagaagccctgtctctacaaaatacagagagaaaaaatcagccagtcatggtggcctacacctgtagtcccagcattccgggaggctgaggtgggaggatcacttgagcccagggaggttggggctgcagtgagccatgatcacaccactgcactccagccaggtgacatagcgagatcctgtctaaaaaaataaaaaataaataatggaacacagcaagtcctaggaagtaggttaaaactaattctttaaaaaaaaaaaaaagttgagcctgaattaaatgtaatgtttccaagtgacaggtatccacatttgcatggttacaagccactgccagttagcagtagcactttcctggcactgtggtcggttttgttttgttttgctttgtttagagacggggtctcactttccaggctggcctcaaactcctgcactcaagcaattcttctaccctggcctcccaagtagctggaattacaggtgtgcgccatcacaactagctggtggtcagttttgttactctgagagctgttcacttctctgaattcacctagagtggttggaccatcagatgtttgggcaaaactgaaagctctttgcaaccacacaccttccctgagcttacatcactgcccttttgagcagaaagtctaaattccttccaagacagtagaattccatcccagtaccaaagccagataggccccctaggaaactgaggtaagagcagtctctaaaaactacccacagcagcattggtgcaggggaacttggccattaggttattatttgagaggaaagtcctcacatcaatagtacatatgaaagtgacctccaaggggattggtgaatactcataaggatcttcaggctgaacagactatgtctggggaaagaacggattatgccccattaaataacaagttgtgttcaagagtcagagcagtgagctcagaggcccttctcactgagacagcaacatttaaaccaaaccagaggaagtatttgtggaactcactgcctcagtttgggtaaaggatgagcagacaagtcaactaaagaaaaaagaaaagcaaggaggagggttgagcaatctagagcatggagtttgttaagtgctctctggatttgagttgaagagcatccatttgagttgaaggccacagggcacaatgagctctcccttctaccaccagaaagtccctggtcaggtctcaggtagtgcggtgtggctcagctgggtttttaattagcgcattctctatccaacatttaattgtttgaaagcctccatatagttagattgtgctttgtaattttgttgttgttgctctatcttattgtatatgcattgagtattaacctgaatgttttgttacttaaatattaaaaacactgttatcctacagtt

SEQ ID NO: 35 - protein, 264 aa, Mus musculus
MSVTACQGLGFVVSLIGFAGIIAATCMDQWSTQDLYNNPVTAVFNYQGLWRSCVRESSGFTECRGYFTLLGLPAMLQAVRALMIVGIVLGVIGILVSIFALKCIRIGSMDDSAKAKMTLTSGILFIISGICAIIGVSVFANMLVTNFWMSTANMYSGMGGMGGMVQTVQTRYTFGAALFVGWVAGGLTLIGGVMMCIACRGLTPDDSNFKAVSYHASGQNVAYRPGGFKASTGFGSNTRNKKIYDGGARTEDDEQSHPTKYDYV

SEQ ID NO: 36 - DNA, 2786 bp, Mus musculus
ggccgggaaccttcccagcaagagggtggtggttgctcctggaagcctgcgcccagcagctgaagccatggccaccaccacgtgccaggtggtagggcttctcctgtccctcctgggtctggccggctgcatagccgccactgggatggacatgtggagcactcaagacctgtatgacaacccagtcaccgccgtgttccagtatgaagggctctggaggagttgcgtgcaacagagctcggggttcaccgagtgccggccatacttcaccatcctgggccttccagccatgctgcaagctgtacgagccctgatgatcgtgggcattgttctgggggtcatcggtatcctcgtgtccatcttcgccctgaagtgcattcgcattggtagcatggatgactctgccaaggccaagatgactctgacttctgggatcttgttcatcatctccggcatctgtgcaatcattggtgtgtctgtgtttgccaacatgctggtgaccaacttctggatgtccacagctaacatgtacagcggcatgggcggcatgggtggcatggtgcagaccgttcagaccaggtacaccttcggtgcagctctgttcgtgggctgggttgctggaggcctcaccctgattgggggagtgatgatgtgcatcgcctgccgtggcctgacaccagatgacagcaacttcaaagctgtgtcttaccatgcctctggccaaaatgttgcctacaggcctggaggctttaaggccagcactggctttgggtccaacaccagaaacaagaagatctacgatgggggtgcccgcacagaagacgatgaacagtctcatcctaccaagtatgactatgtgtagtgctctaagacccgccaacctgtgtgcaggaggaacccttccccaagaagagctcaccccaaagcaacgggagtctaccttgttcccttgttgatttcaactgacatctgaaagttggtaaagcctgattttcatccatagggaggctagacagtcttggccacatgtgtctgcctctaaatatcccatcacaaaacagctgagttatcgtttatgagttagaggccataacactcactttagcccaaccctctgctttttaccgtagactttcttttcatctggtgatggaatggaatttgactcacagactaatactttaatggtttagagaaactttccttcctcgtacttaataagcctgctgatggtcgattttccagcttgaccaccaagggaaattttaaaaggaaaaaaaaatacattaaaaggcattatttcctactcaattgtgccttacccacccccaacttgactgataataataatgaacaccacttaaagaaagaatgccagaggaaagatagttgtgtttccccccagccagtcatctgagtccccctatgtggtgatctagaacattactcgccacagtgattttcaaagaaggcaagcgagcctgttcgctctgctcagcatctgctgattccagcaaggcccttccagagctttccactagaagtcctccttctctcggaagtcagaaattccccctagaagagtaagaaatagattcttttgggtaacctgagtcctaggtatagttataataaatagtatattagcaaaacggtttggtatctcagtgaattagtttcagccttacatatagaaaaagctggggaaaaaaaaagcatcccttgacattgtctatagcgtaagatcctatataaatccaagcttcaacaaaagctcactgagtctaatagttttcttttgaggtctccacggccttagtactcatagatgcagcccctgtttaaaagtaaaaaaattaaagtagcttaaaacgggttctttttttttttttttttttcaaaaaatccaatagagacctgtgtgtctggcatagctacagttactgccaatcgacagggccacttctttggtcctgtaggcagttttgcagttctgacagctgcgccgggcatcaatatgcagaccacacccttctctgtgcttgtaggacgacccgttcaaggagaaagcatgaactccatctccatgtgagcctgaatgctcccaggaaatggagatagggtgctctccaaaacccacctgaacctgaaacagctgtagcgctatgctgtaagagcctggccatcaagttcctatggagaaaaagggcagtccttgcattaatagtgcatatataagtggcctctggggggcagggatgaatattcagtggtggctccgagtatgtacagaccgtctaaggagctgtgttgaccaagagccaggttaatacgcagagtttttcccactgggactacagtgattttagactatactgaagaaggccctctggaaaatcattatctgaaatggcataaagaatgaacagaccaaacaatttaaggggagggggcaggtggaaggagggggaaggaggtagaaataagaatctagggcatgaagattgttaaggttcttggggtccaaatggaaggtcacccctttgaggccatggacacaatgcaccccacccctacccccacctgcccacccaccagaaagtccctggtcggactggaggcagtgagaatcagctgttttcagttagtgggtctcggtgtagcacctggctgtttcaaagcttccccttgctttgccgttttttccgccattgctgtcttgttttctgtgttattaacctccatgttttgtacgttaaatattaaaacactgttaacatccattc

SEQ ID NO: 37 - protein, 264 aa, Mus musculus
MATTTCQVVGLLLSLLGLAGCIAATGMDMWSTQDLYDNPVTAVFQYEGLWRSCVQQSSGFTECRPYFTILGLPAMLQAVRALMIVGIVLGVIGILVSIFALKCIRIGSMDDSAKAKMTLTSGILFIISGICAIIGVSVFANMLVTNFWMSTANMYSGMGGMGGMVQTVQTRYTFGAALFVGWVAGGLTLIGGVMMCIACRGLTPDDSNFKAVSYHASGQNVAYRPGGFKASTGFGSNTRNKKIYDGGARTEDDEQSHPTKYDYV

SEQ ID NO: 38 - DNA, 40 bp, Artificial
  Description of artificial sequence: Oligonucleotide
gagaggatcccgtacggtggctgcaccatctgtcttcatc

SEQ ID NO: 39 - DNA, 37 bp, Artificial
  Description of artificial sequence: Oligonucleotide
gagagcggccgcctaacactctcccctgttgaagctc

SEQ ID NO: 40 - DNA, 324 bp, Artificial
  Description of artificial sequence: PCR product
cgtacggtggctgcaccatctgtcttcatcttcccgccatctgatgagcagttgaaatctggaactgcctctgttgtgtgcctgctgaataacttctatcccagagaggccaaagtacagtggaaggtggataacgccctccaatcgggtaactcccaggagagtgtcacagagcaggacagcaaggacagcacctacagcctcagcagcaccctgacgctgagcaaagcagactacgagaaacacaaagtctacgcctgcgaagtcacccatcagggcctgagctcgcccgtcacaaagagcttcaacaggggagagtgttag

SEQ ID NO: 41 - protein, 107 aa, Artificial [sequence omitted]

SEQ ID NO: 42 - DNA, 34 bp, Artificial
  Description of artificial sequence: Oligonucleotide
gagaaagctttccaccaagggcccatcggtcttc

SEQ ID NO: 43 - DNA, 36 bp, Artificial
  Description of artificial sequence: Oligonucleotide
gagagcggccgctcatttacccggagacagggagag

SEQ ID NO: 44 - DNA, 21 bp, Artificial
  Description of artificial sequence: Oligonucleotide
taccagttgaacttgacctca

SEQ ID NO: 45 - DNA, 981 bp, Artificial
  Description of artificial sequence: PCR product
ggcccatcggtcttccccctggcaccctcctccaagagcacctctgggggcacagcggccctgggctgcctggtcaaggactacttccccgaaccggtgacggtgtcgtggaactcaggcgccctgaccagcggcgtgcacaccttcccggctgtcctacagtcctcaggactctactccctcagcagcgtggtgaccgtgccctccagcagcttgggcacccagacctacatctgcaacgtgaatcacaagcccagcaacaccaaggtggacaagaaagttgagcccaaatcttgtgacaaaactcacacatgcccaccgtgcccagcacctgaactcctggggggaccgtcagtcttcctcttccccccaaaacccaaggacaccctcatgatctcccggacccctgaggtcacatgcgtggtggtggacgtgagccacgaagaccctgaggtcaagttcaactggtacgtggacggcgtggaggtgcataatgccaagacaaagccgcgggaggagcagtacaacagcacgtaccgtgtggtcagcgtcctcaccgtcctgcaccaggactggctgaatggcaaggagtacaagtgcaaggtctccaacaaagccctcccagcccccatcgagaaaaccatctccaaagccaaagggcagccccgagaaccacaggtgtacaccctgcccccatcccgggatgagctgaccaagaaccaggtcagcctgacctgcctggtcaaaggcttctatcccagcgacatcgccgtggagtgggagagcaatgggcagccggagaacaactacaagaccacgcctcccgtgctggactccgacggctccttcttcctctatagcaagctcaccgtggacaagagcaggtggcagcaggggaacgtcttctcatgctccgtgatgcatgaggctctgcacaaccactacacgcagaagagcctctccctgtctccgggtaaatga

SEQ ID NO: 46 - protein, 326 aa, Artificial
  Description of artificial sequence: Translation of PCR product
GPSVFPLAPSSKSTSGGTAALGCLVKDYFPEPVTVSWNSGALTSGVHTFPAVLQSSGLYSLSSVVTVPSSSLGTQTYICNVNHKPSNTKVDKKVEPKSCDKTHTCPPCPAPELLGGPSVFLFPPKPKDTLMISRTPEVTCVVVDVSHEDPEVKFNWYVDGVEVHNAKTKPREEQYNSTYRVVSVLTVLHQDWLNGKEYKCKVSNKALPAPIEKTISKAKGQPREPQVYTLPPSRDELTKNQVSLTCLVKGFYPSDIAVEWESNGQPENNYKTTPPVLDSDGSFFLYSKLTVDKSRWQQGNVFSCSVMHEALHNHYTQKSLSLSPGK

SEQ ID NO: 47 - DNA, 32 bp, Artificial
  Description of artificial sequence: Oligonucleotide
  misc_feature (31)..(32): n is a, c, g, or t
ttttttttttttttttttttttttttttttnn

SEQ ID NO: 48 - DNA, 30 bp, Artificial
  Description of artificial sequence: Oligonucleotide
aagcagtggtatcaacgcagagtacgcggg

SEQ ID NO: 49 - DNA, 26 bp, Artificial
  Description of artificial sequence: Oligonucleotide
ctgctcactggatggtgggaagatgg

SEQ ID NO: 50 - DNA, 25 bp, Artificial
  Description of artificial sequence: Oligonucleotide
gggacagtcactgagctgctcagag

SEQ ID NO: 51 - DNA, 25 bp, Artificial
  Description of artificial sequence: Oligonucleotide
acaggggccagtggatagaccgatg

SEQ ID NO: 52 - DNA, 27 bp, Artificial
  Description of artificial sequence: Oligonucleotide
agccagggaccaagggatagacagatg

SEQ ID NO: 53 - DNA, 45 bp, Artificial
  Description of artificial sequence: Oligonucleotide
gtaatacgactcactatagggcaagcagtggtatcaacgcagagt

SEQ ID NO: 54 - DNA, 22 bp, Artificial
  Description of artificial sequence: Oligonucleotide
gtaatacgactcactatagggc

SEQ ID NO: 55 - DNA, 351 bp, Artificial
  Description of artificial sequence: PCR product
caggttcagctgcagcagtctggagctgagctgatgaagcctggggcctcagtgaagatatcctgcaaggctactggctacacattcagtagctactggatagagtgggtaaagcagaggcctggacatggccttgagtggattggagagattttacctggaagtggtagtactaactacaatgagaagttcaagggcaaggccacattcactgcagatacatcctccaacacagcctacatgcaactcagcagcctgacatctgaggactctgccgtctattactgtgcaagatatgattacccctggtttgcttactggggccaagggactctggtcactgtctctgca

SEQ ID NO: 56 - DNA, 354 bp, Artificial
  Description of artificial sequence: PCR product
cagatccagttggtgcagtctggacctgagctgaagaagcctggagagacagtcaagatctcctgcaaggcttctgggtataccttcacaaactatggaatgaactgggtgaagcaggctccaggaaagggtttaaagtggatgggctggataaacaccaacactggagagccaacatatgctgaagagttcaagggacggtttgccttctctttggaaacctctgccagcactgcctatttgcagatcaacaacctcaaaaatgaggacacggctacatatttctgtgcaagactgggttttggtaatgctatggactactggggtcaaggaacctcagtcaccgtctcctca

SEQ ID NO: 57 - DNA, 348 bp, Artificial
  Description of artificial sequence: PCR product
caggttcagctgcagcagtctggagctgagctggcgaggcccggggcttcagtgaagctgtcctgcaaggcttctggctacaccttcactgactactatataaactgggtgaagcagaggactggacagggccttgagtggattggagagatttatcctggaagtggtaatacttactacaatgagaagttcaagggcaaggccacactgactgcagacaaatcctccagcacagcctacatgcagctcagcagcctgacatctgaggactctgcagtctatttctgtgcaagatcgtatggtgcctttgactactggggccaaggcaccactctcacagtctcctca

SEQ ID NO: 58 - DNA, 354 bp, Artificial
  Description of artificial sequence: PCR product
caggtccaactgcagcagcctggggctgagctggtgaggcctggggcttcagtgaagctgtcctgcaaggcttctggctacaccttcaccagctactggataaactgggtgaagcagaggcctggacaaggccttgagtggatcggaaatatttatccttctgatagttatactaactacaatcaaaagttcaaggacaaggccacattgactgtagacaaatcctccagcacagcctacatgcagctcagcagcccgacatctgaggactctgcggtctattactgtacaagatcgtggaggggtaactcctttgactactggggccaaggcaccactctcacagtctcctca

SEQ ID NO: 59 - DNA, 354 bp, Artificial
  Description of artificial sequence: PCR product
caggttcagctgcagcagtctggacctgagctggtgaagcctggggcttcagtgaagatgtcctgcaaggcttctggatacacattcactgactatgttataagctgggtgaagcagagaactggacagggccttgagtggattggagagatttatcctggaagtggtagtacttactacaatgagaagttcaagggcaaggccacactgactgcagacaaatcctccaacacagcctacatgcagctcagcagcctgacatctgaggactctgcggtctatttctgtgcaagaggggtattactacgggctatggactactggggtcaaggaacctcagtcaccgtctcctca

SEQ ID NO: 60 - DNA, 360 bp, Artificial
  Description of artificial sequence: PCR product
caggttcacctacaacagtctggttctgaactgaggagtcctgggtcttcagtaaagctttcatgcaaggattttgattcagaagtcttcccttttgcttatatgagttggattaggcagaagcctgggcatggatttgaatggattggagacatactcccaagtattggtagaacaatctatggagagaagtttgaggacaaagccacactggatgcagacacagtgtccaacacagcctacttggagctcaacagtctgacatctgaggactctgctatctactactgtgcaaggggggagggctacggtgcctggtttgcttactggggccaagggactctggtcactgtctctgca

SEQ ID NO: 61 - DNA, 339 bp, Artificial
  Description of artificial sequence: PCR product
gacattgtgatgacacagtctccatcctccctgactgtgacagcaggagagaaggtcactatgagctgcaagtccagtcagagtctgttaaacagtggaaatcaaaagaactacttgacctggtaccagcagaaaccagggcagcctcctaaactgttgatctactgggcatccactagggaatctggggtccctgatcgcttcacaggcagtggatctggaacagatttcactctcaccatcagcagtgtgcaggctgaagacctggcagtttattactgtcagaatgattatagttatccgctcacgttcggtgctgggaccaagctggagctgaaa

SEQ ID NO: 62 - DNA, 318 bp, Artificial
  Description of artificial sequence: PCR product
caaattgttctcacccagtctccagcaatcatgtctgcatctccaggggagaaggtcaccataacctgcagtgccagctcaagtgtaagttacatgcactggttccagcagaagccaggcacttctcccaaactctggatttatagcacatccaacctggcttctggagtccctgctcgcttcagtggcagtggatctgggacctcttactctctcacaatcagccgaatggaggctgaagatgctgccacttattactgccagcaaaggagtagttacccacccacgttcggaggggggaccaagctggaaataaaa

SEQ ID NO: 63 - DNA, 321 bp, Artificial
  Description of artificial sequence: PCR product
gacattgtgatgacccagtctcaaaaattcatgtccacatcagtaggagacagggtcagcatcacctgcaaggccagtcagaatgttcgtactgctgtagcctggtatcaacagaaaccagggcagtctcctaaagcactgatttacttggcatccaaccggcacactggagtccctgatcgcttcacaggcagtggatctgggacagatttcactctcaccattagcaatgtgcaatctgaagacctggcagattatttctgtctgcaacattggaattatcctctgacgttcggtggaggcaccaagctggaaatcaaa

SEQ ID NO: 64 - DNA, 339 bp, Artificial
  Description of artificial sequence: PCR product
gacattgtgatgtcacagtctccatcctccctagctgtgtcagttggagagaaggttactatgagctgcaagtccagtcagagccttttatatagtagcaatcaaaagaactacttggcctggtaccagcagaaaccagggcagtctcctaaactgctgatttactgggcatccactagggaatctggggtccctgatcgcttcacaggcagtggatctgggacagatttcactctcaccatcagcagtgtgaaggctgaagacctggcagtttattactgtcagcaatattatagctatccgctcacgttcggtgctgggaccaagctggagctgaaa

SEQ ID NO: 65 - DNA, 339 bp, Artificial
  Description of artificial sequence: PCR product
gacattgtgatgacacagtctccatcctccctgactgtgacagcaggagagaaggtcactatgagctgcaagtccagtcagagtctgttaaacagtggaaatcaaaagaactacttgacctggtaccagcagaaaccagggcagcctcctaaactgttgatctactgggcatccactagggaatctggggtccctgatcgcttcacaggcagtggatctggaacagatttcactctcaccatcagcagtgtgcaggctgaagacctggcagtttattactgtcagaatgattatagttatccattcacgttcggctcggggacaaagttggaaataaaa

SEQ ID NO: 66 - DNA, 336 bp, Artificial
  Description of artificial sequence: PCR product
gacattgtgatgtcacagtctccatcctccctggctgtgtcagcaggagagaaggtcactatgagctgcaaatccagtcagagtctgctcaacagtagaacccgaaagaactacttggcttggtaccagcagaaaccagggcagtctcctaaactgctgatctactgggcatccactagggaatctggggtccctgatcgcttcacaggcagtggatctgggacagatttcactctcaccatcagcagtgtgcaggctgaagacctggcagtttattactgcaagcaatcttataatctgtacacgttcggaggggggaccaagctggaaataaaa

SEQ ID NO: 67 - DNA, 339 bp, Artificial
  Description of artificial sequence: PCR product
gacatcgtgatgtcacagtctccatcctccctagctgtgtcagttggagagaaggttactatgagctgcaagtccagtcagagccttttatatagtagcaatcaaaagaactacttggcctggtaccagcagaaaccagggcagtctcctaaactgctgatttactgggcatccactagggaatctggggtccctgatcgcttcacaggcagtggatctgcaacagatttcactctgaccatcagcagtgtgcaggctgaagaccttgcagattatcactgtggacagggttacagctatccgtacacgttcggaggggggaccaagctggaaataaaa

SEQ ID NO: 68 - DNA, 339 bp, Artificial; identical to SEQ ID NO: 64
  Description of artificial sequence: PCR product

SEQ ID NO: 69 - DNA, 321 bp, Artificial
  Description of artificial sequence: PCR product
aacattgtaatgacccaatctcccaaatccatgtccatgtcagtaggagagagggtcaccttgacctgcaaggccagtgagaatgtggttacttatgtttcctggtatcaacagaaaccagagcagtctcctaaactgctgatatacggggcatccaaccggtacactggggtccccgatcgcttcacaggcagtggatctgcaacagatttcactctcaccatcagcagtgtgaaggctgaagacctggcagtttattactgtcagcaatattatagctatccgctcacgttcggtgctgggaccaagctggagctgaaa

SEQ ID NO: 70 - DNA, 43 bp, Artificial
  Description of artificial sequence: Oligonucleotide
gagaaagcttgccgccaccatggaatggacctgggtctttctc

SEQ ID NO: 71 - DNA, 43 bp, Artificial
  Description of artificial sequence: Oligonucleotide
gagagggcccttggtggaggctgcagagacagtgaccagagtc

SEQ ID NO: 72 - DNA, 47 bp, Artificial
  Description of artificial sequence: Oligonucleotide
gagaaagcttgccgccaccatggattggctgtggaacttgctattcc

SEQ ID NO: 73 - DNA, 44 bp, Artificial
  Description of artificial sequence: Oligonucleotide
gagagggcccttggtggaggctgaggagacggtgactgaggttc

SEQ ID NO: 74 - DNA, 46 bp, Artificial
  Description of artificial sequence: Oligonucleotide
gagaaagcttgccgccaccatggaatggatctggatctttctcttc

SEQ ID NO: 75 - DNA, 44 bp, Artificial
  Description of artificial sequence: Oligonucleotide
gagagggcccttggtggaggctgaggagactgtgagagtggtgc

SEQ ID NO: 76 - DNA, 46 bp, Artificial
  Description of artificial sequence: Oligonucleotide
gagaaagcttgccgccaccatgggatggagctgtatcatcctcttc

SEQ ID NO: 77 - DNA, 43 bp, Artificial
  Description of artificial sequence: Oligonucleotide
gagagggcccttggtggaggctgaggagactgtgagagtggtg

SEQ ID NO: 78 - DNA, 47 bp, Artificial
  Description of artificial sequence: Oligonucleotide
gagaaagcttgccgccaccatggaatggaggatctttctcttcatcc

SEQ ID NO: 79 - DNA, 44 bp, Artificial; identical to SEQ ID NO: 73
  Description of artificial sequence: Oligonucleotide

SEQ ID NO: 80 - DNA, 51 bp, Artificial
  Description of artificial sequence: Oligonucleotide
gagaggtctcaagcttagccaccatggactggatttggatcatgctccatc

SEQ ID NO: 81 - DNA, 44 bp, Artificial
  Description of artificial sequence: Oligonucleotide
gagagggcccttggtggaggctgcagagacagtgaccagagtcc

SEQ ID NO: 82 - DNA, 43 bp, Artificial
  Description of artificial sequence: Oligonucleotide
gagaaagcttgccgccaccatggaatcacagactcaggtcctc

SEQ ID NO: 83 - DNA, 34 bp, Artificial
  Description of artificial sequence: Oligonucleotide
cacacgtacgtttcagctccagcttggtcccagc

SEQ ID NO: 84 - DNA, 46 bp, Artificial
  Description of artificial sequence: Oligonucleotide
gagaaagcttgccgccaccatgcattttcaagtgcagattttcagc

SEQ ID NO: 85 - DNA, 30 bp, Artificial
  Description of artificial sequence: Oligonucleotide
cacacgtacgttttatttccagcttggtcc

SEQ ID NO: 86 - DNA, 44 bp, Artificial
  Description of artificial sequence: Oligonucleotide
gagaaagcttgccgccaccatggagtttcagacccaggtctttg

SEQ ID NO: 87 - DNA, 33 bp, Artificial
  Description of artificial sequence: Oligonucleotide
cacacgtacgtttgatttccagcttggtgcctc

SEQ ID NO: 88 - DNA, 46 bp, Artificial
  Description of artificial sequence: Oligonucleotide
gagaaagcttgccgccaccatggattcacaggcccaggttcttatg

SEQ ID NO: 89 - DNA, 30 bp, Artificial
  Description of artificial sequence: Oligonucleotide
cacacgtacgtttcagctccagcttggtcc

SEQ ID NO: 90 - DNA, 46 bp, Artificial
  Description of artificial sequence: Oligonucleotide
gagaaagcttgccgccaccatggaatcacagactcaggtcctcatg

SEQ ID NO: 91 - DNA, 30 bp, Artificial
  Description of artificial sequence: Oligonucleotide
cacacgtacgttttatttccaactttgtcc

SEQ ID NO: 92 - DNA, 49 bp, Artificial
  Description of artificial sequence: Oligonucleotide
gagaaagcttgccgccaccatggattcacaggcccaggttcttatattg

SEQ ID NO: 93 - DNA, 30 bp, Artificial; identical to SEQ ID NO: 85
  Description of artificial sequence: Oligonucleotide

SEQ ID NO: 94 - DNA, 46 bp, Artificial; identical to SEQ ID NO: 88
  Description of artificial sequence: Oligonucleotide

SEQ ID NO: 95 - DNA, 30 bp, Artificial; identical to SEQ ID NO: 85
  Description of artificial sequence: Oligonucleotide

SEQ ID NO: 96 - DNA, 46 bp, Artificial
  Description of artificial sequence: Oligonucleotide
gagaaagcttgccgccaccatggattcacaggctcaggttcttatg

SEQ ID NO: 97 - DNA, 33 bp, Artificial
  Description of artificial sequence: Oligonucleotide
cacacgtacgtttcagctccagcttggtcccag

SEQ ID NO: 98 - DNA, 41 bp, Artificial
  Description of artificial sequence: Oligonucleotide
gagaaagcttagccaccatggaatcacagactctggtcttc

SEQ ID NO: 99 - DNA, 30 bp, Artificial; identical to SEQ ID NO: 89
  Description of artificial sequence: Oligonucleotide

SEQ ID NO: 100 - DNA, 1401 bp, Artificial
  Description of artificial sequence: chimeric monoclonal antibody
atggaatggacctgggtctttctcttcctcctgtcagtaactgcaggtgtccactcccaggttcagctgcagcagtctggagctgagctgatgaagcctggggcctcagtgaagatatcctgcaaggctactggctacacattcagtagctactggatagagtgggtaaagcagaggcctggacatggccttgagtggattggagagattttacctggaagtggtagtactaactacaatgagaagttcaagggcaaggccacattcactgcagatacatcctccaacacagcctacatgcaactcagcagcctgacatctgaggactctgccgtctattactgtgcaagatatgattacccctggtttgcttactggggccaagggactctggtcactgtctctgcagcctccaccaagggcccatcggtcttccccctggcaccctcctccaagagcacctctgggggcacagcggccctgggctgcctggtcaaggactacttccccgaaccggtgacggtgtcgtggaactcaggcgccctgaccagcggcgtgcacaccttcccggctgtcctacagtcctcaggactctactccctcagcagcgtggtgaccgtgccctccagcagcttgggcacccagacctacatctgcaacgtgaatcacaagcccagcaacaccaaggtggacaagaaagttgagcccaaatcttgtgacaaaactcacacatgcccaccgtgcccagcacctgaactcctggggggaccgtcagtcttcctcttccccccaaaacccaaggacaccctcatgatctcccggacccctgaggtcacatgcgtggtggtggacgtgagccacgaagaccctgaggtcaagttcaactggtacgtggacggcgtggaggtgcataatgccaagacaaagccgcgggaggagcagtacaacagcacgtaccgtgtggtcagcgtcctcaccgtcctgcaccaggactggctgaatggcaaggagtacaagtgcaaggtctccaacaaagccctcccagcccccatcgagaaaaccatctccaaagccaaagggcagccccgagaaccacaggtgtacaccctgcccccatcccgggatgagctgaccaagaaccaggtcagcctgacctgcctggtcaaaggcttctatcccagcgacatcgccgtggagtgggagagcaatgggcagccggagaacaactacaagaccacgcctcccgtgctggactccgacggctccttcttcctctatagcaagctcaccgtggacaagagcaggtggcagcaggggaacgtcttctcatgctccgtgatgcatgaggctctgcacaaccactacacgcagaagagcctctccctgtctccgggtaaatga

SEQ ID NO: 101 - DNA, 1404 bp, Artificial
  Description of artificial sequence: chimeric monoclonal antibody
atggattggctgtggaacttgctattcctgatggcagctgcccaaagtatccaagcacagatccagttggtgcagtctggacctgagctgaagaagcctggagagacagtcaagatctcctgcaaggcttctgggtataccttcacaaactatggaatgaactgggtgaagcaggctccaggaaagggtttaaagtggatgggctggataaacaccaacactggagagccaacatatgctgaagagttcaagggacggtttgccttctctttggaaacctctgccagcactgcctatttgcagatcaacaacctcaaaaatgaggacacggctacatatttctgtgcaagactgggttttggtaatgctatggactactggggtcaaggaacctcagtcaccgtctcctcagcctccaccaagggcccatcggtcttccccctggcaccctcctccaagagcacctctgggggcacagcggccctgggctgcctggtcaaggactacttccccgaaccggtgacggtgtcgtggaactcaggcgccctgaccagcggcgtgcacaccttcccggctgtcctacagtcctcaggactctactccctcagcagcgtggtgaccgtgccctccagcagcttgggcacccagacctacatctgcaacgtgaatcacaagcccagcaacaccaaggtggacaagaaagttgagcccaaatcttgtgacaaaactcacacatgcccaccgtgcccagcacctgaactcctggggggaccgtcagtcttcctcttccccccaaaacccaaggacaccctcatgatctcccggacccctgaggtcacatgcgtggtggtggacgtgagccacgaagaccctgaggtcaagttcaactggtacgtggacggcgtggaggtgcataatgccaagacaaagccgcgggaggagcagtacaacagcacgtaccgtgtggtcagcgtcctcaccgtcctgcaccaggactggctgaatggcaaggagtacaagtgcaaggtctccaacaaagccctcccagcccccatcgagaaaaccatctccaaagccaaagggcagccccgagaaccacaggtgtacaccctgcccccatcccgggatgagctgaccaagaaccaggtcagcctgacctgcctggtcaaaggcttctatcccagcgacatcgccgtggagtgggagagcaatgggcagccggagaacaactacaagaccacgcctcccgtgctggactccgacggctccttcttcctctatagcaagctcaccgtggacaagagcaggtggcagcaggggaacgtcttctcatgctccgtgatgcatgaggctctgcacaaccactacacgcagaagagcctctccctgtctccgggtaaatga

SEQ ID NO: 102 - DNA, 1398 bp, Artificial
  Description of artificial sequence: chimeric monoclonal antibody
atggaatggatctggatctttctcttcatcctctcaggaactgcaggtgtccactcccaggttcagctgcagcagtctggagctgagctggcgaggcccggggcttcagtgaagctgtcctgcaaggcttctggctacaccttcactgactactatataaactgggtgaagcagaggactggacagggccttgagtggattggagagatttatcctggaagtggtaatacttactacaatgagaagttcaagggcaaggccacactgactgcagacaaatcctccagcacagcctacatgcagctcagcagcctgacatctgaggactctgcagtctatttctgtgcaagatcgtatggtgcctttgactactggggccaaggcaccactctcacagtctcctcagcctccaccaagggcccatcggtcttccccctggcaccctcctccaagagcacctctgggggcacagcggccctgggctgcctggtcaaggactacttccccgaaccggtgacggtgtcgtggaactcaggcgccctgaccagcggcgtgcacaccttcccggctgtcctacagtcctcaggactctactccctcagcagcgtggtgaccgtgccctccagcagcttgggcacccagacctacatctgcaacgtgaatcacaagcccagcaacaccaaggtggacaagaaagttgagcccaaatcttgtgacaaaactcacacatgcccaccgtgcccagcacctgaactcctggggggaccgtcagtcttcctcttccccccaaaacccaaggacaccctcatgatctcccggacccctgaggtcacatgcgtggtggtggacgtgagccacgaagaccctgaggtcaagttcaactggtacgtggacggcgtggaggtgcataatgccaagacaaagccgcgggaggagcagtacaacagcacgtaccgtgtggtcagcgtcctcaccgtcctgcaccaggactggctgaatggcaaggagtacaagtgcaaggtctccaacaaagccctcccagcccccatcgagaaaaccatctccaaagccaaagggcagccccgagaaccacaggtgtacaccctgcccccatcccgggatgagctgaccaagaaccaggtcagcctgacctgcctggtcaaaggcttctatcccagcgacatcgccgtggagtgggagagcaatgggcagccggagaacaactacaagaccacgcctcccgtgctggactccgacggctccttcttcctctatagcaagctcaccgtggacaagagcaggtggcagcaggggaacgtcttctcatgctccgtgatgcatgaggctctgcacaaccactacacgcagaagagcctctccctgtctccgggtaaatga

SEQ ID NO: 103 - DNA, 1404 bp, Artificial
  Description of artificial sequence: chimeric monoclonal antibody
atgggatggagctgtatcatcctcttcttggtagcaacagctacaggtgtccactcccaggtccaactgcagcagcctggggctgagctggtgaggcctggggcttcagtgaagctgtcctgcaaggcttctggctacaccttcaccagctactggataaactgggtgaagcagaggcctggacaaggccttgagtggatcggaaatatttatccttctgatagttatactaactacaatcaaaagttcaaggacaaggccacattgactgtagacaaatcctccagcacagcctacatgcagctcagcagcccgacatctgaggactctgcggtctattactgtacaagatcgtggaggggtaactcctttgactactggggccaaggcaccactctcacagtctcctcagcctccaccaagggcccatcggtcttccccctggcaccctcctccaagagcacctctgggggcacagcggccctgggctgcctggtcaaggactacttccccgaaccggtgacggtgtcgtggaactcaggcgccctgaccagcggcgtgcacaccttcccggctgtcctacagtcctcaggactctactccctcagcagcgtggtgaccgtgccctccagcagcttgggcacccagacctacatctgcaacgtgaatcacaagcccagcaacaccaaggtggacaagaaagttgagcccaaatcttgtgacaaaactcacacatgcccaccgtgcccagcacctgaactcctggggggaccgtcagtcttcctcttccccccaaaacccaaggacaccctcatgatctcccggacccctgaggtcacatgcgtggtggtggacgtgagccacgaagaccctgaggtcaagttcaactggtacgtggacggcgtggaggtgcataatgccaagacaaagccgcgggaggagcagtacaacagcacgtaccgtgtggtcagcgtcctcaccgtcctgcaccaggactggctgaatggcaaggagtacaagtgcaaggtctccaacaaagccctcccagcccccatcgagaaaaccatctccaaagccaaagggcagccccgagaaccacaggtgtacaccctgcccccatcccgggatgagctgaccaagaaccaggtcagcctgacctgcctggtcaaaggcttctatcccagcgacatcgccgtggagtgggagagcaatgggcagccggagaacaactacaagaccacgcctcccgtgctggactccgacggctccttcttcctctatagcaagctcaccgtggacaagagcaggtggcagcaggggaacgtcttctcatgctccgtgatgcatgaggctctgcacaaccactacacgcagaagagcctctccctgtctccgggtaaatga

SEQ ID NO: 104 - DNA, 1401 bp, Artificial
  Description of artificial sequence: chimeric monoclonal antibody
atggaatggaggatctttctcttcatcctgtcaggaactgcaggtgtccactcccaggttcagctgcagcagtctggacctgagctggtgaagcctggggcttcagtgaagatgtcctgcaaggcttctggatacacattcactgactatgttataagctgggtgaagcagagaactggacagggccttgagtggattggagagatttatcctggaagtggtagtacttactacaatgagaagttcaagggcaaggccacactgactgcagacaaatcctccaacacagcctacatgcagctcagcagcctgacatctgaggactctgcggtctatttctgtgcaagaggggtattactacgggctatggactactggggtcaaggaacctcagtcaccgtctcctcagcctccaccaagggcccatcggtcttccccctggcaccctcctccaagagcacctctgggggcacagcggccctgggctgcctggtcaaggactacttccccgaaccggtgacggtgtcgtggaactcaggcgccctgaccagcggcgtgcacaccttcccggctgtcctacagtcctcaggactctactccctcagcagcgtggtgaccgtgccctccagcagcttgggcacccagacctacatctgcaacgtgaatcacaagcccagcaacaccaaggtggacaagaaagttgagcccaaatcttgtgacaaaactcacacatgcccaccgtgcccagcacctgaactcctggggggaccgtcagtcttcctcttccccccaaaacccaaggacaccctcatgatctcccggacccctgaggtcacatgcgtggtggtggacgtgagccacgaagaccctgaggtcaagttcaactggtacgtggacggcgtggaggtgcataatgccaagacaaagccgcgggaggagcagtacaacagcacgtaccgtgtggtcagcgtcctcaccgtcctgcaccaggactggctgaatggcaaggagtacaagtgcaaggtctccaacaaagccctcccagcccccatcgagaaaaccatctccaaagccaaagggcagccccgagaaccacaggtgtacaccctgcccccatcccgggatgagctgaccaagaaccaggtcagcctgacctgcctggtcaaaggcttctatcccagcgacatcgccgtggagtgggagagcaatgggcagccggagaacaactacaagaccacgcctcccgtgctggactccgacggctccttcttcctctatagcaagctcaccgtggacaagagcaggtggcagcaggggaacgtcttctcatgctccgtgatgcatgaggctctgcacaaccactacacgcagaagagcctctccctgtctccgggtaaatga

SEQ ID NO: 105 - DNA, 1410 bp, Artificial
  Description of artificial sequence: chimeric monoclonal antibody
atggactggatttggatcatgctccatctgctggcagcagctacaggtatccaatcccaggttcacctacaacagtctggttctgaactgaggagtcctgggtcttcagtaaagctttcatgcaaggattttgattcagaagtcttcccttttgcttatatgagttggattaggcagaagcctgggcatggatttgaatggattggagacatactcccaagtattggtagaacaatctatggagagaagtttgaggacaaagccacactggatgcagacacagtgtccaacacagcctacttggagctcaacagtctgacatctgaggactctgctatctactactgtgcaaggggggagggctacggtgcctggtttgcttactggggccaagggactctggtcactgtctctgcagcctccaccaagggcccatcggtcttccccctggcaccctcctccaagagcacctctgggggcacagcggccctgggctgcctggtcaaggactacttccccgaaccggtgacggtgtcgtggaactcaggcgccctgaccagcggcgtgcacaccttcccggctgtcctacagtcctcaggactctactccctcagcagcgtggtgaccgtgccctccagcagcttgggcacccagacctacatctgcaacgtgaatcacaagcccagcaacaccaaggtggacaagaaagttgagcccaaatcttgtgacaaaactcacacatgcccaccgtgcccagcacctgaactcctggggggaccgtcagtcttcctcttccccccaaaacccaaggacaccctcatgatctcccggacccctgaggtcacatgcgtggtggtggacgtgagccacgaagaccctgaggtcaagttcaactggtacgtggacggcgtggaggtgcataatgccaagacaaagccgcgggaggagcagtacaacagcacgtaccgtgtggtcagcgtcctcaccgtcctgcaccaggactggctgaatggcaaggagtacaagtgcaaggtctccaacaaagccctcccagcccccatcgagaaaaccatctccaaagccaaagggcagccccgagaaccacaggtgtacaccctgcccccatcccgggatgagctgaccaagaaccaggtcagcctgacctgcctggtcaaaggcttctatcccagcgacatcgccgtggagtgggagagcaatgggcagccggagaacaactacaagaccacgcctcccgtgctggactccgacggctccttcttcctctatagcaagctcaccgtggacaagagcaggtggcagcaggggaacgtcttctcatgctccgtgatgcatgaggctctgcacaaccactacacgcagaagagcctctccctgtctccgggtaaatga

SEQ ID NO: 106 - DNA, 723 bp, Artificial
  Description of artificial sequence: chimeric monoclonal antibody
atggaatcacagactcaggtcctcatgtccctgctgttctgggtatctggtacctgtggggacattgtgatgacacagtctccatcctccctgactgtgacagcaggagagaaggtcactatgagctgcaagtccagtcagagtctgttaaacagtggaaatcaaaagaactacttgacctggtaccagcagaaaccagggcagcctcctaaactgttgatctactgggcatccactagggaatctggggtccctgatcgcttcacaggcagtggatctggaacagatttcactctcaccatcagcagtgtgcaggctgaagacctggcagtttattactgtcagaatgattatagttatccgctcacgttcggtgctgggaccaagctggagctgaaacgtacggtggctgcaccatctgtcttcatcttcccgccatctgatgagcagttgaaatctggaactgcctctgttgtgtgcctgctgaataacttctatcccagagaggccaaagtacagtggaaggtggataacgccctccaatcgggtaactcccaggagagtgtcacagagcaggacagcaaggacagcacctacagcctcagcagcaccctgacgctgagcaaagcagactacgagaaacacaaagtctacgcctgcgaagtcacccatcagggcctgagctcgcccgtcacaaagagcttcaacaggggagagtgttag

SEQ ID NO: 107 - DNA, 708 bp, Artificial
  Description of artificial sequence: chimeric monoclonal antibody
atgcattttcaagtgcagattttcagcttcctgctaatcagtgcctcagtcataatgtccagaggacaaattgttctcacccagtctccagcaatcatgtctgcatctccaggggagaaggtcaccataacctgcagtgccagctcaagtgtaagttacatgcactggttccagcagaagccaggcacttctcccaaactctggatttatagcacatccaacctggcttctggagtccctgctcgcttcagtggcagtggatctgggacctcttactctctcacaatcagccgaatggaggctgaagatgctgccacttattactgccagcaaaggagtagttacccacccacgttcggaggggggaccaagctggaaataaaacgtacggtggctgcaccatctgtcttcatcttcccgccatctgatgagcagttgaaatctggaactgcctctgttgtgtgcctgctgaataacttctatcccagagaggccaaagtacagtggaaggtggataacgccctccaatcgggtaactcccaggagagtgtcacagagcaggacagcaaggacagcacctacagcctcagcagcaccctgacgctgagcaaagcagactacgagaaacacaaagtctacgcctgcgaagtcacccatcagggcctgagctcgcccgtcacaaagagcttcaacaggggagagtgttag

SEQ ID NO: 108 - DNA, 705 bp, Artificial
  Description of artificial sequence: chimeric monoclonal antibody
atggagtttcagacccaggtctttgtattcgtgttgctctggttgtctggtgttgatggagacattgtgatgacccagtctcaaaaattcatgtccacatcagtaggagacagggtcagcatcacctgcaaggccagtcagaatgttcgtactgctgtagcctggtatcaacagaaaccagggcagtctcctaaagcactgatttacttggcatccaaccggcacactggagtccctgatcgcttcacaggcagtggatctgggacagatttcactctcaccattagcaatgtgcaatctgaagacctggcagattatttctgtctgcaacattggaattatcctctgacgttcggtggaggcaccaagctggaaatcaaacgtacggtggctgcaccatctgtcttcatcttcccgccatctgatgagcagttgaaatctggaactgcctctgttgtgtgcctgctgaataacttctatcccagagaggccaaagtacagtggaaggtggataacgccctccaatcgggtaactcccaggagagtgtcacagagcaggacagcaaggacagcacctacagcctcagcagcaccctgacgctgagcaaagcagactacgagaaacacaaagtctacgcctgcgaagtcacccatcagggcctgagctcgcccgtcacaaagagcttcaacaggggagagtgttag

SEQ ID NO: 109 - DNA, 723 bp, Artificial
  Description of artificial sequence: chimeric monoclonal antibody
atggattcacaggcccaggttcttatgttactgctgctatgggtatctggtacctgtggggacattgtgatgtcacagtctccatcctccctagctgtgtcagttggagagaaggttactatgagctgcaagtccagtcagagccttttatatagtagcaatcaaaagaactacttggcctggtaccagcagaaaccagggcagtctcctaaactgctgatttactgggcatccactagggaatctggggtccctgatcgcttcacaggcagtggatctgggacagatttcactctcaccatcagcagtgtgaaggctgaagacctggcagtttattactgtcagcaatattatagctatccgctcacgttcggtgctgggaccaagctggagctgaaacgtacggtggctgcaccatctgtcttcatcttcccgccatctgatgagcagttgaaatctggaactgcctctgttgtgtgcctgctgaataacttctatcccagagaggccaaagtacagtggaaggtggataacgccctccaatcgggtaactcccaggagagtgtcacagagcaggacagcaaggacagcacctacagcctcagcagcaccctgacgctgagcaaagcagactacgagaaacacaaagtctacgcctgcgaagtcacccatcagggcctgagctcgcccgtcacaaagagcttcaacaggggagagtgttag

SEQ ID NO: 110 - DNA, 723 bp, Artificial
  Description of artificial sequence: chimeric monoclonal antibody
atggaatcacagactcaggtcctcatgtccctgctgttctgggtatctggtacctgtggggacattgtgatgacacagtctccatcctccctgactgtgacagcaggagagaaggtcactatgagctgcaagtccagtcagagtctgttaaacagtggaaatcaaaagaactacttgacctggtaccagcagaaaccagggcagcctcctaaactgttgatctactgggcatccactagggaatctggggtccctgatcgcttcacaggcagtggatctggaacagatttcactctcaccatcagcagtgtgcaggctgaagacctggcagtttattactgtcagaatgattatagttatccattcacgttcggctcggggacaaagttggaaataaaacgtacggtggctgcaccatctgtcttcatcttcccgccatctgatgagcagttgaaatctggaactgcctctgttgtgtgcctgctgaataacttctatcccagagaggccaaagtacagtggaaggtggataacgccctccaatcgggtaactcccaggagagtgtcacagagcaggacagcaaggacagcacctacagcctcagcagcaccctgacgctgagcaaagcagactacgagaaacacaaagtctacgcctgcgaagtcacccatcagggcctgagctcgcccgtcacaaagagcttcaacaggggagagtgttag

SEQ ID NO: 111 - DNA, 720 bp, Artificial
  Description of artificial sequence: chimeric monoclonal antibody
atggattcacaggcccaggttcttatattgctgctgctatgggtatctggtacctgtggggacattgtgatgtcacagtctccatcctccctggctgtgtcagcaggagagaaggtcactatgagctgcaaatccagtcagagtctgctcaacagtagaacccgaaagaactacttggcttggtaccagcagaaaccagggcagtctcctaaactgctgatctactgggcatccactagggaatctggggtccctgatcgcttcacaggcagtggatctgggacagatttcactctcaccatcagcagtgtgcaggctgaagacctggcagtttattactgcaagcaatcttataatctgtacacgttcggaggggggaccaagctggaaataaaacgtacggtggctgcaccatctgtcttcatcttcccgccatctgatgagcagttgaaatctggaactgcctctgttgtgtgcctgctgaataacttctatcccagagaggccaaagtacagtggaaggtggataacgccctccaatcgggtaactcccaggagagtgtcacagagcaggacagcaaggacagcacctacagcctcagcagcaccctgacgctgagcaaagcagactacgagaaacacaaagtctacgcctgcgaagtcacccatcagggcctgagctcgcccgtcacaaagagcttcaacaggggagagtgttag

SEQ ID NO: 112 - DNA, 723 bp, Artificial
  Description of artificial sequence: chimeric monoclonal antibody
atggattcacaggcccaggttcttatgttactgctgctatgggtatctggtacctgtggggacatcgtgatgtcacagtctccatcctccctagctgtgtcagttggagagaaggttactatgagctgcaagtccagtcagagccttttatatagtagcaatcaaaagaactacttggcctggtaccagcagaaaccagggcagtctcctaaactgctgatttactgggcatccactagggaatctggggtccctgatcgcttcacaggcagtggatctgcaacagatttcactctgaccatcagcagtgtgcaggctgaagaccttgcagattatcactgtggacagggttacagctatccgtacacgttcggaggggggaccaagctggaaataaaacgtacggtggctgcaccatctgtcttcatcttcccgccatctgatgagcagttgaaatctggaactgcctctgttgtgtgcctgctgaataacttctatcccagagaggccaaagtacagtggaaggtggataacgccctccaatcgggtaactcccaggagagtgtcacagagcaggacagcaaggacagcacctacagcctcagcagcaccctgacgctgagcaaagcagactacgagaaacacaaagtctacgcctgcgaagtcacccatcagggcctgagctcgcccgtcacaaagagcttcaacaggggagagtgttag

SEQ ID NO: 113 - DNA, 723 bp, Artificial
  Description of artificial sequence: chimeric monoclonal antibody
atggattcacaggctcaggttcttatgttactgctgctatgggtatctggtacctgtggggacattgtgatgtcacagtctccatcctccctagctgtgtcagttggagagaaggttactatgagctgcaagtccagtcagagccttttatatagtagcaatcaaaagaactacttggcctggtaccagcagaaaccagggcagtctcctaaactgctgatttactgggcatccactagggaatctggggtccctgatcgcttcacaggcagtggatctgggacagatttcactctcaccatcagcagtgtgaaggctgaagacctggcagtttattactgtcagcaatattatagctatccgctcacgttcggtgctgggaccaagctggagctgaaacgtacggtggctgcaccatctgtcttcatcttcccgccatctgatgagcagttgaaatctggaactgcctctgttgtgtgcctgctgaataacttctatcccagagaggccaaagtacagtggaaggtggataacgccctccaatcgggtaactcccaggagagtgtcacagagcaggacagcaaggacagcacctacagcctcagcagcaccctgacgctgagcaaagcagactacgagaaacacaaagtctacgcctgcgaagtcacccatcagggcctgagctcgcccgtcacaaagagcttcaacaggggagagtgttag

SEQ ID NO: 114 - DNA, 705 bp, Artificial
  Description of artificial sequence: chimeric monoclonal antibody
atggaatcacagactctggtcttcatatccatactgctctggttatatggagctgatgggaacattgtaatgacccaatctcccaaatccatgtccatgtcagtaggagagagggtcaccttgacctgcaaggccagtgagaatgtggttacttatgtttcctggtatcaacagaaaccagagcagtctcctaaactgctgatatacggggcatccaaccggtacactggggtccccgatcgcttcacaggcagtggatctgcaacagatttcactctcaccatcagcagtgtgaaggctgaagacctggcagtttattactgtcagcaatattatagctatccgctcacgttcggtgctgggaccaagctggagctgaaacgtacggtggctgcaccatctgtcttcatcttcccgccatctgatgagcagttgaaatctggaactgcctctgttgtgtgcctgctgaataacttctatcccagagaggccaaagtacagtggaaggtggataacgccctccaatcgggtaactcccaggagagtgtcacagagcaggacagcaaggacagcacctacagcctcagcagcaccctgacgctgagcaaagcagactacgagaaacacaaagtctacgcctgcgaagtcacccatcagggcctgagctcgcccgtcacaaagagcttcaacaggggagagtgttag

SEQ ID NO: 115 - protein, 466 aa, Artificial
  Description of artificial sequence: chimeric monoclonal antibody
MEWTWVFLFLLSVTAGVHSQVQLQQSGAELMKPGASVKISCKATGYTFSSYWIEWVKQRPGHGLEWIGEILPGSGSTNYNEKFKGKATFTADTSSNTAYMQLSSLTSEDSAVYYCARYDYPWFAYWGQGTLVTVSAASTKGPSVFPLAPSSKSTSGGTAALGCLVKDYFPEPVTVSWNSGALTSGVHTFPAVLQSSGLYSLSSVVTVPSSSLGTQTYICNVNHKPSNTKVDKKVEPKSCDKTHTCPPCPAPELLGGPSVFLFPPKPKDTLMISRTPEVTCVVVDVSHEDPEVKFNWYVDGVEVHNAKTKPREEQYNSTYRVVSVLTVLHQDWLNGKEYKCKVSNKALPAPIEKTISKAKGQPREPQVYTLPPSRDELTKNQVSLTCLVKGFYPSDIAVEWESNGQPENNYKTTPPVLDSDGSFFLYSKLTVDKSRWQQGNVFSCSVMHEALHNHYTQKSLSLSPGK

SEQ ID NO: 116 - protein, 467 aa, Artificial
  Description of artificial sequence: chimeric monoclonal antibody
MDWLWNLLFLMAAAQSIQAQIQLVQSGPELKKPGETVKISCKASGYTFTNYGMNWVKQAPGKGLKWMGWINTNTGEPTYAEEFKGRFAFSLETSASTAYLQINNLKNEDTATYFCARLGFGNAMDYWGQGTSVTVSSASTKGPSVFPLAPSSKSTSGGTAALGCLVKDYFPEPVTVSWNSGALTSGVHTFPAVLQSSGLYSLSSVVTVPSSSLGTQTYICNVNHKPSNTKVDKKVEPKSCDKTHTCPPCPAPELLGGPSVFLFPPKPKDTLMISRTPEVTCVVVDVSHEDPEVKFNWYVDGVEVHNAKTKPREEQYNSTYRVVSVLTVLHQDWLNGKEYKCKVSNKALPAPIEKTISKAKGQPREPQVYTLPPSRDELTKNQVSLTCLVKGFYPSDIAVEWESNGQPENNYKTTPPVLDSDGSFFLYSKLTVDKSRWQQGNVFSCSVMHEALHNHYTQKSLSLSPGK

SEQ ID NO: 117 - protein, 465 aa, Artificial
  Description of artificial sequence: chimeric monoclonal antibody
MEWIWIFLFILSGTAGVHSQVQLQQSGAELARPGASVKLSCKASGYTFTDYYINWVKQRTGQGLEWIGEIYPGSGNTYYNEKFKGKATLTADKSSSTAYMQLSSLTSEDSAVYFCARSYGAFDYWGQGTTLTVSSASTKGPSVFPLAPSSKSTSGGTAALGCLVKDYFPEPVTVSWNSGALTSGVHTFPAVLQSSGLYSLSSVVTVPSSSLGTQTYICNVNHKPSNTKVDKKVEPKSCDKTHTCPPCPAPELLGGPSVFLFPPKPKDTLMISRTPEVTCVVVDVSHEDPEVKFNWYVDGVEVHNAKTKPREEQYNSTYRVVSVLTVLHQDWLNGKEYKCKVSNKALPAPIEKTISKAKGQPREPQVYTLPPSRDELTKNQVSLTCLVKGFYPSDIAVEWESNGQPENNYKTTPPVLDSDGSFFLYSKLTVDKSRWQQGNVFSCSVMHEALHNHYTQKSLSLSPGK

SEQ ID NO: 118 - protein, 467 aa, Artificial
  Description of artificial sequence: chimeric monoclonal antibody
MGWSCIILFLVATATGVHSQVQLQQPGAELVRPGASVKLSCKASGYTFTSYWINWVKQRPGQGLEWIGNIYPSDSYTNYNQKFKDKATLTVDKSSSTAYMQLSSPTSEDSAVYYCTRSWRGNSFDYWGQGTTLTVSSASTKGPSVFPLAPSSKSTSGGTAALGCLVKDYFPEPVTVSWNSGALTSGVHTFPAVLQSSGLYSLSSVVTVPSSSLGTQTYICNVNHKPSNTKVDKKVEPKSCDKTHTCPPCPAPELLGGPSVFLFPPKPKDTLMISRTPEVTCVVVDVSHEDPEVKFNWYVDGVEVHNAKTKPREEQYNSTYRVVSVLTVLHQDWLNGKEYKCKVSNKALPAPIEKTISKAKGQPREPQVYTLPPSRDELTKNQVSLTCLVKGFYPSDIAVEWESNGQPENNYKTTPPVLDSDGSFFLYSKLTVDKSRWQQGNVFSCSVMHEALHNHYTQKSLSLSPGK

SEQ ID NO: 119 - protein, 466 aa, Artificial
  Description of artificial sequence: chimeric monoclonal antibody
MEWRIFLFILSGTAGVHSQVQLQQSGPELVKPGASVKMSCKASGYTFTDYVISWVKQRTGQGLEWIGEIYPGSGSTYYNEKFKGKATLTADKSSNTAYMQLSSLTSEDSAVYFCARGVLLRAMDYWGQGTSVTVSSASTKGPSVFPLAPSSKSTSGGTAALGCLVKDYFPEPVTVSWNSGALTSGVHTFPAVLQSSGLYSLSSVVTVPSSSLGTQTYICNVNHKPSNTKVDKKVEPKSCDKTHTCPPCPAPELLGGPSVFLFPPKPKDTLMISRTPEVTCVVVDVSHEDPEVKFNWYVDGVEVHNAKTKPREEQYNSTYRVVSVLTVLHQDWLNGKEYKCKVSNKALPAPIEKTISKAKGQPREPQVYTLPPSRDELTKNQVSLTCLVKGFYPSDIAVEWESNGQPENNYKTTPPVLDSDGSFFLYSKLTVDKSRWQQGNVFSCSVMHEALHNHYTQKSLSLSPGK

SEQ ID NO: 120 - protein, 469 aa, Artificial [sequence omitted]

SEQ ID NO: 121 - protein, 240 aa, Artificial
  Description of artificial sequence: chimeric monoclonal antibody
MESQTQVLMSLLFWVSGTCGDIVMTQSPSSLTVTAGEKVTMSCKSSQSLLNSGNQKNYLTWYQQKPGQPPKLLIYWASTRESGVPDRFTGSGSGTDFTLTISSVQAEDLAVYYCQNDYSYPLTFGAGTKLELKRTVAAPSVFIFPPSDEQLKSGTASVVCLLNNFYPREAKVQWKVDNALQSGNSQESVTEQDSKDSTYSLSSTLTLSKADYEKHKVYACEVTHQGLSSPVTKSFNRGEC

SEQ ID NO: 122 - protein, 235 aa, Artificial
  Description of artificial sequence: chimeric monoclonal antibody
MHFQVQIFSFLLISASVIMSRGQIVLTQSPAIMSASPGEKVTITCSASSSVSYMHWFQQKPGTSPKLWIYSTSNLASGVPARFSGSGSGTSYSLTISRMEAEDAATYYCQQRSSYPPTFGGGTKLEIKRTVAAPSVFIFPPSDEQLKSGTASVVCLLNNFYPREAKVQWKVDNALQSGNSQESVTEQDSKDSTYSLSSTLTLSKADYEKHKVYACEVTHQGLSSPVTKSFNRGEC

SEQ ID NO: 123 - protein, 234 aa, Artificial
  Description of artificial sequence: chimeric monoclonal antibody
MEFQTQVFVFVLLWLSGVDGDIVMTQSQKFMSTSVGDRVSITCKASQNVRTAVAWYQQKPGQSPKALIYLASNRHTGVPDRFTGSGSGTDFTLTISNVQSEDLADYFCLQHWNYPLTFGGGTKLEIKRTVAAPSVFIFPPSDEQLKSGTASVVCLLNNFYPREAKVQWKVDNALQSGNSQESVTEQDSKDSTYSLSSTLTLSKADYEKHKVYACEVTHQGLSSPVTKSFNRGEC

SEQ ID NO: 124 - protein, 240 aa, Artificial
  Description of artificial sequence: chimeric monoclonal antibody
MDSQAQVLMLLLLWVSGTCGDIVMSQSPSSLAVSVGEKVTMSCKSSQSLLYSSNQKNYLAWYQQKPGQSPKLLIYWASTRESGVPDRFTGSGSGTDFTLTISSVKAEDLAVYYCQQYYSYPLTFGAGTKLELKRTVAAPSVFIFPPSDEQLKSGTASVVCLLNNFYPREAKVQWKVDNALQSGNSQESVTEQDSKDSTYSLSSTLTLSKADYEKHKVYACEVTHQGLSSPVTKSFNRGEC

SEQ ID NO: 125 - protein, 240 aa, Artificial
  Description of artificial sequence: chimeric monoclonal antibody
MESQTQVLMSLLFWVSGTCGDIVMTQSPSSLTVTAGEKVTMSCKSSQSLLNSGNQKNYLTWYQQKPGQPPKLLIYWASTRESGVPDRFTGSGSGTDFTLTISSVQAEDLAVYYCQNDYSYPFTFGSGTKLEIKRTVAAPSVFIFPPSDEQLKSGTASVVCLLNNFYPREAKVQWKVDNALQSGNSQESVTEQDSKDSTYSLSSTLTLSKADYEKHKVYACEVTHQGLSSPVTKSFNRGEC

SEQ ID NO: 126 - protein, 239 aa, Artificial
  Description of artificial sequence: chimeric monoclonal antibody
MDSQAQVLILLLLWVSGTCGDIVMSQSPSSLAVSAGEKVTMSCKSSQSLLNSRTRKNYLAWYQQKPGQSPKLLIYWASTRESGVPDRFTGSGSGTDFTLTISSVQAEDLAVYYCKQSYNLYTFGGGTKLEIKRTVAAPSVFIFPPSDEQLKSGTASVVCLLNNFYPREAKVQWKVDNALQSGNSQESVTEQDSKDSTYSLSSTLTLSKADYEKHKVYACEVTHQGLSSPVTKSFNRGEC

SEQ ID NO: 127 - protein, 240 aa, Artificial
  Description of artificial sequence: chimeric monoclonal antibody
MDSQAQVLMLLLLWVSGTCGDIVMSQSPSSLAVSVGEKVTMSCKSSQSLLYSSNQKNYLAWYQQKPGQSPKLLIYWASTRESGVPDRFTGSGSATDFTLTISSVQAEDLADYHCGQGYSYPYTFGGGTKLEIKRTVAAPSVFIFPPSDEQLKSGTASVVCLLNNFYPREAKVQWKVDNALQSGNSQESVTEQDSKDSTYSLSSTLTLSKADYEKHKVYACEVTHQGLSSPVTKSFNRGEC

SEQ ID NO: 128 - protein, 240 aa, Artificial; identical to SEQ ID NO: 124
  Description of artificial sequence: chimeric monoclonal antibody

SEQ ID NO: 129 - protein, 234 aa, Artificial
  Description of artificial sequence: chimeric monoclonal antibody
MESQTLVFISILLWLYGADGNIVMTQSPKSMSMSVGERVTLTCKASENVVTYVSWYQQKPEQSPKLLIYGASNRYTGVPDRFTGSGSATDFTLTISSVKAEDLAVYYCQQYYSYPLTFGAGTKLELKRTVAAPSVFIFPPSDEQLKSGTASVVCLLNNFYPREAKVQWKVDNALQSGNSQESVTEQDSKDSTYSLSSTLTLSKADYEKHKVYACEVTHQGLSSPVTKSFNRGEC

SEQ ID NO: 130 - DNA, 18 bp, Artificial
  Description of artificial sequence: Oligonucleotide
ccaagggctatggcgttc

SEQ ID NO: 131 - DNA, 18 bp, Artificial
  Description of artificial sequence: Oligonucleotide
ccgaaggtgtacctggtc

SEQ ID NO: 132 - protein, 117 aa, Artificial
  Description of artificial sequence: Translation of PCR product
QVQLQQSGAELMKPGASVKISCKATGYTFSSYWIEWVKQRPGHGLEWIGEILPGSGSTNYNEKFKGKATFTADTSSNTAYMQLSSLTSEDSAVYYCARYDYPWFAYWGQGTLVTVSA

SEQ ID NO: 133 - protein, 118 aa, Artificial
  Description of artificial sequence: Translation of PCR product
QIQLVQSGPELKKPGETVKISCKASGYTFTNYGMNWVKQAPGKGLKWMGWINTNTGEPTYAEEFKGRFAFSLETSASTAYLQINNLKNEDTATYFCARLGFGNAMDYWGQGTSVTVSS

SEQ ID NO: 134 - protein, 116 aa, Artificial
  Description of artificial sequence: Translation of PCR product
QVQLQQSGAELARPGASVKLSCKASGYTFTDYYINWVKQRTGQGLEWIGEIYPGSGNTYYNEKFKGKATLTADKSSSTAYMQLSSLTSEDSAVYFCARSYGAFDYWGQGTTLTVSS

SEQ ID NO: 135 - protein, 118 aa, Artificial
  Description of artificial sequence: Translation of PCR product
QVQLQQPGAELVRPGASVKLSCKASGYTFTSYWINWVKQRPGQGLEWIGNIYPSDSYTNYNQKFKDKATLTVDKSSSTAYMQLSSPTSEDSAVYYCTRSWRGNSFDYWGQGTTLTVSS

SEQ ID NO: 136 - protein, 118 aa, Artificial
  Description of artificial sequence: Translation of PCR product
QVQLQQSGPELVKPGASVKMSCKASGYTFTDYVISWVKQRTGQGLEWIGEIYPGSGSTYYNEKFKGKATLTADKSSNTAYMQLSSLTSEDSAVYFCARGVLLRAMDYWGQGTSVTVSS

SEQ ID NO: 137 - protein, 120 aa, Artificial
  Description of artificial sequence: Translation of PCR product
QVHLQQSGSELRSPGSSVKLSCKDFDSEVFPFAYMSWIRQKPGHGFEWIGDILPSIGRTIYGEKFEDKATLDADTVSNTAYLELNSLTSEDSAIYYCARGEGYGAWFAYWGQGTLVTVSA

SEQ ID NO: 138 - protein, 113 aa, Artificial
  Description of artificial sequence: Translation of PCR product
DIVMTQSPSSLTVTAGEKVTMSCKSSQSLLNSGNQKNYLTWYQQKPGQPPKLLIYWASTRESGVPDRFTGSGSGTDFTLTISSVQAEDLAVYYCQNDYSYPLTFGAGTKLELK

SEQ ID NO: 139 - protein, 106 aa, Artificial
  Description of artificial sequence: Translation of PCR product
QIVLTQSPAIMSASPGEKVTITCSASSSVSYMHWFQQKPGTSPKLWIYSTSNLASGVPARFSGSGSGTSYSLTISRMEAEDAATYYCQQRSSYPPTFGGGTKLEIK

SEQ ID NO: 140 - protein, 107 aa, Artificial
  Description of artificial sequence: Translation of PCR product
DIVMTQSQKFMSTSVGDRVSITCKASQNVRTAVAWYQQKPGQSPKALIYLASNRHTGVPDRFTGSGSGTDFTLTISNVQSEDLADYFCLQHWNYPLTFGGGTKLEIK

SEQ ID NO: 141 - protein, 113 aa, Artificial
  Description of artificial sequence: Translation of PCR product
DIVMSQSPSSLAVSVGEKVTMSCKSSQSLLYSSNQKNYLAWYQQKPGQSPKLLIYWASTRESGVPDRFTGSGSGTDFTLTISSVKAEDLAVYYCQQYYSYPLTFGAGTKLELK

SEQ ID NO: 142 - protein, 113 aa, Artificial
  Description of artificial sequence: Translation of PCR product
DIVMTQSPSSLTVTAGEKVTMSCKSSQSLLNSGNQKNYLTWYQQKPGQPPKLLIYWASTRESGVPDRFTGSGSGTDFTLTISSVQAEDLAVYYCQNDYSYPFTFGSGTKLEIK

SEQ ID NO: 143 - protein, 112 aa, Artificial
  Description of artificial sequence: Translation of PCR product
DIVMSQSPSSLAVSAGEKVTMSCKSSQSLLNSRTRKNYLAWYQQKPGQSPKLLIYWASTRESGVPDRFTGSGSGTDFTLTISSVQAEDLAVYYCKQSYNLYTFGGGTKLEIK

SEQ ID NO: 144 - protein, 113 aa, Artificial
  Description of artificial sequence: Translation of PCR product
DIVMSQSPSSLAVSVGEKVTMSCKSSQSLLYSSNQKNYLAWYQQKPGQSPKLLIYWASTRESGVPDRFTGSGSATDFTLTISSVQAEDLADYHCGQGYSYPYTFGGGTKLEIK

SEQ ID NO: 145 - protein, 113 aa, Artificial; identical to SEQ ID NO: 141
  Description of artificial sequence: Translation of PCR product

SEQ ID NO: 146 - protein, 107 aa, Artificial
  Description of artificial sequence: Translation of PCR product
NIVMTQSPKSMSMSVGERVTLTCKASENVVTYVSWYQQKPEQSPKLLIYGASNRYTGVPDRFTGSGSATDFTLTISSVKAEDLAVYYCQQYYSYPLTFGAGTKLELK

SEQ ID NO: 147 - DNA, 324 bp, Artificial
  Description of artificial sequence: codon optimized nucleic acid
cgtacggtggccgctcccagcgtgttcatcttcccccccagcgacgagcagctgaagtccggcaccgccagcgtggtgtgcctgctgaacaacttctacccccgggaggccaaggtgcagtggaaggtggacaacgccctgcagagcggcaacagccaggagagcgtcaccgagcaggacagcaaggactccacctacagcctgagcagcaccctgaccctgagcaaggccgactacgagaagcacaaggtgtacgcctgcgaggtgacccaccagggcctgtccagccccgtgaccaagagcttcaacaggggcgagtgctag

SEQ ID NO: 148 - protein, 107 aa, Artificial [sequence omitted]

SEQ ID NO: 149 - DNA, 981 bp, Artificial
  Description of artificial sequence: codon optimized nucleic acid
ggcccaagcgtgttccccctggcccccagcagcaagagcaccagcggcggcacagccgccctgggctgcctggtgaaggactacttccccgagcccgtgaccgtgagctggaacagcggagccctgacctccggcgtgcacaccttccccgccgtgctgcagagcagcggcctgtacagcctgagcagcgtggtgaccgtgcccagcagcagcctgggcacccagacctacatctgcaacgtgaaccacaagcccagcaacaccaaggtggacaagagagtggagcccaagagctgcgacaagacccacacctgccccccctgcccagccccagagctgctgggcggacccagcgtgttcctgttcccccccaagcccaaggacaccctgatgatcagcaggacccccgaggtgacctgcgtggtggtggacgtgagccacgaggacccagaggtgaagttcaactggtacgtggacggcgtggaggtgcacaacgccaagaccaagcccagagaggagcagtacaacagcacctacagggtggtgtccgtgctgaccgtgctgcaccaggactggctgaacggcaaggaatacaagtgcaaggtctccaacaaggccctgccagcccccatcgaaaagaccatcagcaaggccaagggccagccacgggagccccaggtgtacaccctgccccccagccgggaggagatgaccaagaaccaggtgtccctgacctgtctggtgaagggcttctaccccagcgacatcgccgtggagtgggagagcaacggccagcccgagaacaactacaagaccacccccccagtgctggacagcgacggcagcttcttcctgtacagcaagctgaccgtggacaagtccaggtggcagcagggcaacgtgttcagctgcagcgtgatgcacgaggccctgcacaaccactacacccagaagtccctgagcctgagccccggcaagtag

SEQ ID NO: 150 - protein, 326 aa, Artificial
  Description of artificial sequence: codon optimized protein
GPSVFPLAPSSKSTSGGTAALGCLVKDYFPEPVTVSWNSGALTSGVHTFPAVLQSSGLYSLSSVVTVPSSSLGTQTYICNVNHKPSNTKVDKRVEPKSCDKTHTCPPCPAPELLGGPSVFLFPPKPKDTLMISRTPEVTCVVVDVSHEDPEVKFNWYVDGVEVHNAKTKPREEQYNSTYRVVSVLTVLHQDWLNGKEYKCKVSNKALPAPIEKTISKAKGQPREPQVYTLPPSREEMTKNQVSLTCLVKGFYPSDIAVEWESNGQPENNYKTTPPVLDSDGSFFLYSKLTVDKSRWQQGNVFSCSVMHEALHNHYTQKSLSLSPGK

SEQ ID NO: 151 - protein, 15 aa, Artificial
  Epitope
MDQWSTQDLYNNPVT

SEQ ID NO: 152 - protein, 15 aa, Artificial
  Epitope
STQDLYNNPVTAVFN

SEQ ID NO: 153 - protein, 15 aa, Artificial
  Epitope
LYNNPVTAVFNYQGL

SEQ ID NO: 154 - protein, 15 aa, Artificial
  Epitope
PVTAVFNYQGLWRSC

SEQ ID NO: 155 - protein, 15 aa, Artificial
  Epitope
VFNYQGLWRSCVRES

SEQ ID NO: 156 - protein, 15 aa, Artificial
  Epitope
QGLWRSCVRESSGFT

SEQ ID NO: 157 - protein, 15 aa, Artificial
  Epitope
RSCVRESSGFTECRG